European Patent Specification EP 3 559 278 B1, published August 14, 2024. Title: Universal Biosensor for Analyte Detection. Applicant: Fundamental Solutions Corporation. The sequence listing filed with the application follows.

SEQUENCE LISTING (19 sequences)

SEQ ID NO: 1 - DNA, 1929 bp, Artificial Sequence
  Chimeric Protein:  BBP-IgM
  CDS (1)..(1929)
atggtgctgcagacgcaagtgtttatctccctgctgctctggatcagcggagcgtacggcacttacaagctggtgatcaacggtaaaaccttgaagggtgagaccaccactgaggcagtcgacgccgccactgccgagaaggtctttaaacagtatgccaatgataacggcgtggacggcgagtggacctacgatgacgccactaagacattcactgtgactgaaaagcccgaggtgattgacgcgtccgaattgacacctgcggtgaccacctacaaactggttatcaacggcaagactctgaagggcgagaccaccacagaggcagtcgatgccgccaccgccgagaaggtcttcaagcaatatgccaacgacaacggggtggacggggagtggacctacgatgatgccaccaagaccttcaccgtgaccgagaagcccgaagtgatcgatgcgagtgaactgactcccgccgtgacaggttctgcttctggttctggtggttcagcatcagcaccaactttgtttccacttgtctcatgtgagaactcgccatcggatacctcgagcgtagcggtcggatgtctcgctcaagactttcttccggacagcatcacgttttcatggaagtataagaacaattcggatatttcgagcacgcgaggatttcccagcgtattgagagggggaaagtacgcggcaacaagccaggtgctgctcccaagcaaggatgtgatgcagggcactgacgagcatgtagtatgcaaggtacagcaccccaatggaaacaaggaaaagaatgtccctctgcctgtaattgccgagctccctcctaaagtgtcagtgttcgtgccgcccagagatgggttctttggaaacccgcgatcgaagtcgaaactgatctgccaggccacgggattcagccctcggcagattcaagtgtcgtggttgcgggagggaaaacaggtgggatcgggggtgaccacagaccaggtgcaggcggaggctaaagaaagcggtcccaccacatataaggtcacttccacccttactattaaggaatcggattggttgtcacagtcgatgttcacatgtagagtcgatcatcgcggactcacgtttcaacagaacgcgtcatcaatgtgtgtacccgatcaagatacggcgatcagagtattcgccattccgcctagcttcgcatccatttttctcaccaaaagcacaaagctgacatgtcttgtgacagacctcacaacgtacgattcagtcacaatttcatggaccaggcagaatggggaggcggtaaagacgcacaccaacatttcggaaagccatcccaacgccacgttttcggcggtcggggaggcatcgatttgtgaggacgattggaattcaggggagcgcttcacatgcacggtcactcacacggatctcccatccccgttgaagcagacaatctcgcgacccaaaggtgtcgcactgcacaggcccgacgtctacctcctgcctcctgccagggaacagctcaacctccgggaatcagcaacgatcacgtgtcttgtaaccgggttttcaccggctgacgtctttgtccaatggatgcagcggggacaacccttgtcaccagagaagtatgtgacatcagcgcccatgcccgagccacaggctccgggtaggtattttgcccattccatcctcactgtgtccgaggaagagtggaacaccggcgaaacgtacacgtgcgtcgtagcacacgaagcgttgcccaatagagtgactgagagaactgtagataagtccactgagggcgaagtaagcgcggatgaagaaggtttcgaaaacttgtgggctacagcgagcacgtttatcgtgttgttcttgctttcactcttctactccacaactgtaaccctgttcaaggtcaagtag

SEQ ID NO: 2 - protein, 642 aa, Artificial Sequence
  Synthetic Construct
MVLQTQVFISLLLWISGAYGTYKLVINGKTLKGETTTEAVDAATAEKVFKQYANDNGVDGEWTYDDATKTFTVTEKPEVIDASELTPAVTTYKLVINGKTLKGETTTEAVDAATAEKVFKQYANDNGVDGEWTYDDATKTFTVTEKPEVIDASELTPAVTGSASGSGGSASAPTLFPLVSCENSPSDTSSVAVGCLAQDFLPDSITFSWKYKNNSDISSTRGFPSVLRGGKYAATSQVLLPSKDVMQGTDEHVVCKVQHPNGNKEKNVPLPVIAELPPKVSVFVPPRDGFFGNPRSKSKLICQATGFSPRQIQVSWLREGKQVGSGVTTDQVQAEAKESGPTTYKVTSTLTIKESDWLSQSMFTCRVDHRGLTFQQNASSMCVPDQDTAIRVFAIPPSFASIFLTKSTKLTCLVTDLTTYDSVTISWTRQNGEAVKTHTNISESHPNATFSAVGEASICEDDWNSGERFTCTVTHTDLPSPLKQTISRPKGVALHRPDVYLLPPAREQLNLRESATITCLVTGFSPADVFVQWMQRGQPLSPEKYVTSAPMPEPQAPGRYFAHSILTVSEEEWNTGETYTCVVAHEALPNRVTERTVDKSTEGEVSADEEGFENLWATASTFIVLFLLSLFYSTTVTLFKVK

SEQ ID NO: 3 - DNA, 1884 bp, Artificial Sequence
  Chimeric Protein:  BBP-IgAB
  CDS (1)..(1884)
atgccgggtggacccggagtgctccaggcattgcctgcaaccatcttcctgctgttcttgttgtccgccgtctaccttggacctggttgccaggcaacttacaagctggtgatcaacggtaaaaccttgaagggtgagaccaccactgaggcagtcgacgccgccactgccgagaaggtctttaaacagtatgccaatgataacggcgtggacggcgagtggacctacgatgacgccactaagacattcactgtgactgaaaagcccgaggtgattgacgcgtccgaattgacacctgcggtgaccacctacaaactggttatcaacggcaagactctgaagggcgagaccaccacagaggcagtcgatgccgccaccgccgagaaggtcttcaagcaatatgccaacgacaacggggtggacggggagtggacctacgatgatgccaccaagaccttcaccgtgaccgagaagcccgaagtgatcgatgcgagtgaactgactcccgccgtgacaggttctgcttcgggctcaggactgtggatgcataaggtgcctgcatcgctcatggtgagcctgggcgaagatgcacattttcagtgtccccataacagctccaacaacgcgaacgtgacctggtggcgggtgctccatggcaattacacctggccgcctgaatttctcggaccgggagaggacccgaatgggacccttatcatccagaacgtgaataagtcccacggaggaatctacgtctgccgcgtgcaagagggaaatgagagctaccaacagtcatgcggaacgtacctccgcgtccggcagccaccaccgaggccgttcctcgatatgggagagggaactaagaaccggatcattaccgccgaaggcatcatcctcctcttctgcgccgtcgtgccggggactctgcttctgttccggaaaaggtggcaaaacgaaaagctgggtctggacgctggggacgaatacgaggatgaaaacttgtacgagggcctgaatctggacgattgctcgatgtatgaggacattagcagaggactgcagggtacctaccaagacgtgggaagcctgaacatcggggatgtgcagctcgagaaaccaaggaaaagaagagctagcgaaggacgcggatcactgcttacttgcggcgatgtcgaagaaaatcccggaccaatggccagattggcgctgtcgccggtcccttcgcactggatggtggccctgctgctcttgctttcggcggctgagccggtgccagcggctagatcggaggaccgctacagaaatccgaagggttccgcttgctcacgcatctggcaatcaccacgcttcatcgcgcgcaaacgcggcttcactgtcaagatgcactgctatatgaactcggccagcgggaatgtgtcgtggctgtggaagcaggaaatggacgagaatccgcagcaactgaaactggagaagggccggatggaagaatcccagaatgagtcgctggccacccttactatccaaggtatccggtttgaagataacgggatctacttctgtcaacagaagtgtaacaacacttcagaggtgtaccagggatgcggcaccgaactccgcgtcatgggattctccaccctcgcccaactgaagcagcgcaacacgctgaaggacggcatcattatgatccagaccctgctgatcatcctgttcatcattgtgccgatctttctgctcttggataaggacgactcgaaagccggaatggaagaggaccacacgtacgaaggtctggacatcgaccaaactgcgacttacgaggacattgtgaccctccggactggcgaagtcaagtggtccgtgggtgaacaccctggacaggaatag

SEQ ID NO: 4 - protein, 627 aa, Artificial Sequence
  Synthetic Construct
MPGGPGVLQALPATIFLLFLLSAVYLGPGCQATYKLVINGKTLKGETTTEAVDAATAEKVFKQYANDNGVDGEWTYDDATKTFTVTEKPEVIDASELTPAVTTYKLVINGKTLKGETTTEAVDAATAEKVFKQYANDNGVDGEWTYDDATKTFTVTEKPEVIDASELTPAVTGSASGSGLWMHKVPASLMVSLGEDAHFQCPHNSSNNANVTWWRVLHGNYTWPPEFLGPGEDPNGTLIIQNVNKSHGGIYVCRVQEGNESYQQSCGTYLRVRQPPPRPFLDMGEGTKNRIITAEGIILLFCAVVPGTLLLFRKRWQNEKLGLDAGDEYEDENLYEGLNLDDCSMYEDISRGLQGTYQDVGSLNIGDVQLEKPRKRRASEGRGSLLTCGDVEENPGPMARLALSPVPSHWMVALLLLLSAAEPVPAARSEDRYRNPKGSACSRIWQSPRFIARKRGFTVKMHCYMNSASGNVSWLWKQEMDENPQQLKLEKGRMEESQNESLATLTIQGIRFEDNGIYFCQQKCNNTSEVYQGCGTELRVMGFSTLAQLKQRNTLKDGIIMIQTLLIILFIIVPIFLLLDKDDSKAGMEEDHTYEGLDIDQTATYEDIVTLRTGEVKWSVGEHPGQE

SEQ ID NO: 5 - DNA, 936 bp, Artificial Sequence
  Chimeric Protein:  BBP-CD3Z
  CDS (1)..(936)
atgaagtggaaggcgcttttcaccgcggccatcctgcaggcacagttgccgattacagaggcaacttacaagctggtgatcaacggtaaaaccttgaagggtgagaccaccactgaggcagtcgacgccgccactgccgagaaggtctttaaacagtatgccaatgataacggcgtggacggcgagtggacctacgatgacgccactaagacattcactgtgactgaaaagcccgaggtgattgacgcgtccgaattgacacctgcggtgaccacctacaaactggttatcaacggcaagactctgaagggcgagaccaccacagaggcagtcgatgccgccaccgccgagaaggtcttcaagcaatatgccaacgacaacggggtggacggggagtggacctacgatgatgccaccaagaccttcaccgtgaccgagaagcccgaagtgatcgatgcgagtgaactgactcccgccgtgacaggttctgcttctggttctggtcagagctttggcctgctggatcccaaactctgctacctgctggatggaatcctcttcatctatggtgtcattctcactgccttgttcctgagagtgaagttcagcaggagcgcagacgcccccgcgtaccagcagggccagaaccagctctataacgagctcaatctaggacgaagagaggagtacgatgttttggacaagagacgtggccgggaccctgagatggggggaaagccgcagagaaggaagaaccctcaggaaggcctgtacaatgaactgcagaaagataagatggcggaggcctacagtgagattgggatgaaaggcgagcgccggaggggcaaggggcacgatggcctttaccagggtctcagtacagccaccaaggacacctacgacgcccttcacatgcaggccctgccccctcgctaa

SEQ ID NO: 6 - protein, 311 aa, Artificial Sequence
  Synthetic Construct
MKWKALFTAAILQAQLPITEATYKLVINGKTLKGETTTEAVDAATAEKVFKQYANDNGVDGEWTYDDATKTFTVTEKPEVIDASELTPAVTTYKLVINGKTLKGETTTEAVDAATAEKVFKQYANDNGVDGEWTYDDATKTFTVTEKPEVIDASELTPAVTGSASGSGQSFGLLDPKLCYLLDGILFIYGVILTALFLRVKFSRSADAPAYQQGQNQLYNELNLGRREEYDVLDKRRGRDPEMGGKPQRRKNPQEGLYNELQKDKMAEAYSEIGMKGERRRGKGHDGLYQGLSTATKDTYDALHMQALPPR

SEQ ID NO: 7 - DNA, 2340 bp, Artificial Sequence
  Chimeric Protein:  FcgammaR1-IgM
  CDS (1)..(2340)
atgattcttaccagctttggagatgacatgtggcttctaacaactctgctactttgggttccagtcggtggggaagtggttaatgccaccaaggctgtgatcaccttgcagcctccatgggtcagtattttccagaaggaaaatgtcactttatggtgtgaggggcctcacctgcctggagacagttccacacaatggtttatcaacggaacagccgttcagatctccacgcctagttatagcatcccagaggccagttttcaggacagtggcgaatacaggtgtcagataggttcctcaatgccaagtgaccctgtgcagttgcaaatccacaatgattggctgctactccaggcctcccgcagagtcctcacagaaggagaacccctggccttgaggtgtcacggatggaagaataaactggtgtacaatgtggttttctatagaaatggaaaatcctttcagttttcttcagattcggaggtcgccattctgaaaaccaacctgagtcacagcggcatctaccactgctcaggcacgggaagacaccgctacacatctgcaggagtgtccatcacggtgaaagagctgtttaccacgccagtgctgagagcatccgtgtcatctcccttcccggaggggagtctggtcaccctgaactgtgagacgaatttgctcctgcagagacccggcttacagcttcacttctccttctacgtgggcagcaagatcctggagtacaggaacacatcctcagagtaccatatagcaagggcggaaagagaagatgctggattctactggtgtgaggtagccacggaggacagcagtgtccttaagcgcagccctgagttggagctccaagtgcttggtccccagtcatcagctcctggttctgcttctggttctggtggttcagcatcagcaccaactttgtttccacttgtctcatgtgagaactcgccatcggatacctcgagcgtagcggtcggatgtctcgctcaagactttcttccggacagcatcacgttttcatggaagtataagaacaattcggatatttcgagcacgcgaggatttcccagcgtattgagagggggaaagtacgcggcaacaagccaggtgctgctcccaagcaaggatgtgatgcagggcactgacgagcatgtagtatgcaaggtacagcaccccaatggaaacaaggaaaagaatgtccctctgcctgtaattgccgagctccctcctaaagtgtcagtgttcgtgccgcccagagatgggttctttggaaacccgcgatcgaagtcgaaactgatctgccaggccacgggattcagccctcggcagattcaagtgtcgtggttgcgggagggaaaacaggtgggatcgggggtgaccacagaccaggtgcaggcggaggctaaagaaagcggtcccaccacatataaggtcacttccacccttactattaaggaatcggattggttgtcacagtcgatgttcacatgtagagtcgatcatcgcggactcacgtttcaacagaacgcgtcatcaatgtgtgtacccgatcaagatacggcgatcagagtattcgccattccgcctagcttcgcatccatttttctcaccaaaagcacaaagctgacatgtcttgtgacagacctcacaacgtacgattcagtcacaatttcatggaccaggcagaatggggaggcggtaaagacgcacaccaacatttcggaaagccatcccaacgccacgttttcggcggtcggggaggcatcgatttgtgaggacgattggaattcaggggagcgcttcacatgcacggtcactcacacggatctcccatccccgttgaagcagacaatctcgcgacccaaaggtgtcgcactgcacaggcccgacgtctacctcctgcctcctgccagggaacagctcaacctccgggaatcagcaacgatcacgtgtcttgtaaccgggttttcaccggctgacgtctttgtccaatggatgcagcggggacaacccttgtcaccagagaagtatgtgacatcagcgcccatgcccgagccacaggctccgggtaggtattttgcccattccatcctcactgtgtccgaggaagagtggaacaccggcgaaacgtacacgtgcgtcgtagcacacgaagcgttgcccaatagagtgactgagagaactgtagataagtccactgagggcgaagtaagcgcggatgaagaaggtttcgaaaacttgtgggctacagcgagcacgtttatcgtgttgttcttgctttcactcttctactccacaactgtaaccctgttcaaggtcaagtag

SEQ ID NO: 8 - protein, 779 aa, Artificial Sequence
  Synthetic Construct
MILTSFGDDMWLLTTLLLWVPVGGEVVNATKAVITLQPPWVSIFQKENVTLWCEGPHLPGDSSTQWFINGTAVQISTPSYSIPEASFQDSGEYRCQIGSSMPSDPVQLQIHNDWLLLQASRRVLTEGEPLALRCHGWKNKLVYNVVFYRNGKSFQFSSDSEVAILKTNLSHSGIYHCSGTGRHRYTSAGVSITVKELFTTPVLRASVSSPFPEGSLVTLNCETNLLLQRPGLQLHFSFYVGSKILEYRNTSSEYHIARAEREDAGFYWCEVATEDSSVLKRSPELELQVLGPQSSAPGSASGSGGSASAPTLFPLVSCENSPSDTSSVAVGCLAQDFLPDSITFSWKYKNNSDISSTRGFPSVLRGGKYAATSQVLLPSKDVMQGTDEHVVCKVQHPNGNKEKNVPLPVIAELPPKVSVFVPPRDGFFGNPRSKSKLICQATGFSPRQIQVSWLREGKQVGSGVTTDQVQAEAKESGPTTYKVTSTLTIKESDWLSQSMFTCRVDHRGLTFQQNASSMCVPDQDTAIRVFAIPPSFASIFLTKSTKLTCLVTDLTTYDSVTISWTRQNGEAVKTHTNISESHPNATFSAVGEASICEDDWNSGERFTCTVTHTDLPSPLKQTISRPKGVALHRPDVYLLPPAREQLNLRESATITCLVTGFSPADVFVQWMQRGQPLSPEKYVTSAPMPEPQAPGRYFAHSILTVSEEEWNTGETYTCVVAHEALPNRVTERTVDKSTEGEVSADEEGFENLWATASTFIVLFLLSLFYSTTVTLFKVK

SEQ ID NO: 9 - DNA, 2259 bp, Artificial Sequence
  Chimeric Protein:  FcgammaR1-IgAB
  CDS (1)..(2259)
atgattcttaccagctttggagatgacatgtggcttctaacaactctgctactttgggttccagtcggtggggaagtggttaatgccaccaaggctgtgatcaccttgcagcctccatgggtcagtattttccagaaggaaaatgtcactttatggtgtgaggggcctcacctgcctggagacagttccacacaatggtttatcaacggaacagccgttcagatctccacgcctagttatagcatcccagaggccagttttcaggacagtggcgaatacaggtgtcagataggttcctcaatgccaagtgaccctgtgcagttgcaaatccacaatgattggctgctactccaggcctcccgcagagtcctcacagaaggagaacccctggccttgaggtgtcacggatggaagaataaactggtgtacaatgtggttttctatagaaatggaaaatcctttcagttttcttcagattcggaggtcgccattctgaaaaccaacctgagtcacagcggcatctaccactgctcaggcacgggaagacaccgctacacatctgcaggagtgtccatcacggtgaaagagctgtttaccacgccagtgctgagagcatccgtgtcatctcccttcccggaggggagtctggtcaccctgaactgtgagacgaatttgctcctgcagagacccggcttacagcttcacttctccttctacgtgggcagcaagatcctggagtacaggaacacatcctcagagtaccatatagcaagggcggaaagagaagatgctggattctactggtgtgaggtagccacggaggacagcagtgtccttaagcgcagccctgagttggagctccaagtgcttggtccccagtcatcagctcctggttctgcttcgggctcaggactgtggatgcataaggtgcctgcatcgctcatggtgagcctgggcgaagatgcacattttcagtgtccccataacagctccaacaacgcgaacgtgacctggtggcgggtgctccatggcaattacacctggccgcctgaatttctcggaccgggagaggacccgaatgggacccttatcatccagaacgtgaataagtcccacggaggaatctacgtctgccgcgtgcaagagggaaatgagagctaccaacagtcatgcggaacgtacctccgcgtccggcagccaccaccgaggccgttcctcgatatgggagagggaactaagaaccggatcattaccgccgaaggcatcatcctcctcttctgcgccgtcgtgccggggactctgcttctgttccggaaaaggtggcaaaacgaaaagctgggtctggacgctggggacgaatacgaggatgaaaacttgtacgagggcctgaatctggacgattgctcgatgtatgaggacattagcagaggactgcagggtacctaccaagacgtgggaagcctgaacatcggggatgtgcagctcgagaaaccaaggaaaagaagagctagcgaaggacgcggatcactgcttacttgcggcgatgtcgaagaaaatcccggaccaatggccagattggcgctgtcgccggtcccttcgcactggatggtggccctgctgctcttgctttcggcggctgagccggtgccagcggctagatcggaggaccgctacagaaatccgaagggttccgcttgctcacgcatctggcaatcaccacgcttcatcgcgcgcaaacgcggcttcactgtcaagatgcactgctatatgaactcggccagcgggaatgtgtcgtggctgtggaagcaggaaatggacgagaatccgcagcaactgaaactggagaagggccggatggaagaatcccagaatgagtcgctggccacccttactatccaaggtatccggtttgaagataacgggatctacttctgtcaacagaagtgtaacaacacttcagaggtgtaccagggatgcggcaccgaactccgcgtcatgggattctccaccctcgcccaactgaagcagcgcaacacgctgaaggacggcatcattatgatccagaccctgctgatcatcctgttcatcattgtgccgatctttctgctcttggataaggacgactcgaaagccggaatggaagaggaccacacgtacgaaggtctggacatcgaccaaactgcgacttacgaggacattgtgaccctccggactggcgaagtcaagtggtccgtgggtgaacaccctggacaggaatag

SEQ ID NO: 10 - protein, 752 aa, Artificial Sequence
  Synthetic Construct
MILTSFGDDMWLLTTLLLWVPVGGEVVNATKAVITLQPPWVSIFQKENVTLWCEGPHLPGDSSTQWFINGTAVQISTPSYSIPEASFQDSGEYRCQIGSSMPSDPVQLQIHNDWLLLQASRRVLTEGEPLALRCHGWKNKLVYNVVFYRNGKSFQFSSDSEVAILKTNLSHSGIYHCSGTGRHRYTSAGVSITVKELFTTPVLRASVSSPFPEGSLVTLNCETNLLLQRPGLQLHFSFYVGSKILEYRNTSSEYHIARAEREDAGFYWCEVATEDSSVLKRSPELELQVLGPQSSAPGSASGSGLWMHKVPASLMVSLGEDAHFQCPHNSSNNANVTWWRVLHGNYTWPPEFLGPGEDPNGTLIIQNVNKSHGGIYVCRVQEGNESYQQSCGTYLRVRQPPPRPFLDMGEGTKNRIITAEGIILLFCAVVPGTLLLFRKRWQNEKLGLDAGDEYEDENLYEGLNLDDCSMYEDISRGLQGTYQDVGSLNIGDVQLEKPRKRRASEGRGSLLTCGDVEENPGPMARLALSPVPSHWMVALLLLLSAAEPVPAARSEDRYRNPKGSACSRIWQSPRFIARKRGFTVKMHCYMNSASGNVSWLWKQEMDENPQQLKLEKGRMEESQNESLATLTIQGIRFEDNGIYFCQQKCNNTSEVYQGCGTELRVMGFSTLAQLKQRNTLKDGIIMIQTLLIILFIIVPIFLLLDKDDSKAGMEEDHTYEGLDIDQTATYEDIVTLRTGEVKWSVGEHPGQE

SEQ ID NO: 11 - DNA, 1335 bp, Artificial Sequence
  Chimeric Protein:  FcgammaR1-CD3Z
  CDS (1)..(1335)
atgaagtggaaggcgcttttcaccgcggccatcctgcaggcacagttgccgattacagaggcagaagtggttaatgccaccaaggctgtgatcaccttgcagcctccatgggtcagtattttccagaaggaaaatgtcactttatggtgtgaggggcctcacctgcctggagacagttccacacaatggtttatcaacggaacagccgttcagatctccacgcctagttatagcatcccagaggccagttttcaggacagtggcgaatacaggtgtcagataggttcctcaatgccaagtgaccctgtgcagttgcaaatccacaatgattggctgctactccaggcctcccgcagagtcctcacagaaggagaacccctggccttgaggtgtcacggatggaagaataaactggtgtacaatgtggttttctatagaaatggaaaatcctttcagttttcttcagattcggaggtcgccattctgaaaaccaacctgagtcacagcggcatctaccactgctcaggcacgggaagacaccgctacacatctgcaggagtgtccatcacggtgaaagagctgtttaccacgccagtgctgagagcatccgtgtcatctcccttcccggaggggagtctggtcaccctgaactgtgagacgaatttgctcctgcagagacccggcttacagcttcacttctccttctacgtgggcagcaagatcctggagtacaggaacacatcctcagagtaccatatagcaagggcggaaagagaagatgctggattctactggtgtgaggtagccacggaggacagcagtgtccttaagcgcagccctgagttggagctccaagtgcttggtccccagtcatcagctcctggttctgcttctggttctggtcagagctttggcctgctggatcccaaactctgctacctgctggatggaatcctcttcatctatggtgtcattctcactgccttgttcctgagagtgaagttcagcaggagcgcagacgcccccgcgtaccagcagggccagaaccagctctataacgagctcaatctaggacgaagagaggagtacgatgttttggacaagagacgtggccgggaccctgagatggggggaaagccgcagagaaggaagaaccctcaggaaggcctgtacaatgaactgcagaaagataagatggcggaggcctacagtgagattgggatgaaaggcgagcgccggaggggcaaggggcacgatggcctttaccagggtctcagtacagccaccaaggacacctacgacgcccttcacatgcaggccctgccccctcgctaa

SEQ ID NO: 12 - protein, 444 aa, Artificial Sequence
  Synthetic Construct
MKWKALFTAAILQAQLPITEAEVVNATKAVITLQPPWVSIFQKENVTLWCEGPHLPGDSSTQWFINGTAVQISTPSYSIPEASFQDSGEYRCQIGSSMPSDPVQLQIHNDWLLLQASRRVLTEGEPLALRCHGWKNKLVYNVVFYRNGKSFQFSSDSEVAILKTNLSHSGIYHCSGTGRHRYTSAGVSITVKELFTTPVLRASVSSPFPEGSLVTLNCETNLLLQRPGLQLHFSFYVGSKILEYRNTSSEYHIARAEREDAGFYWCEVATEDSSVLKRSPELELQVLGPQSSAPGSASGSGQSFGLLDPKLCYLLDGILFIYGVILTALFLRVKFSRSADAPAYQQGQNQLYNELNLGRREEYDVLDKRRGRDPEMGGKPQRRKNPQEGLYNELQKDKMAEAYSEIGMKGERRRGKGHDGLYQGLSTATKDTYDALHMQALPPR

SEQ ID NO: 13 - DNA, 1848 bp, Artificial Sequence
  Chimeric Protein:  FcgammaR1-IgE
  CDS (1)..(1848)
catatggaagtggttaatgccaccaaggctgtgatcaccttgcagcctccatgggtcagtattttccagaaggaaaatgtcactttatggtgtgaggggcctcacctgcctggagacagttccacacaatggtttatcaacggaacagccgttcagatctccacgcctagttatagcatcccagaggccagttttcaggacagtggcgaatacaggtgtcagataggttcctcaatgccaagtgaccctgtgcagttgcaaatccacaatgattggctgctactccaggcctcccgcagagtcctcacagaaggagaacccctggccttgaggtgtcacggatggaagaataaactggtgtacaatgtggttttctatagaaatggaaaatcctttcagttttcttcagattcggaggtcgccattctgaaaaccaacctgagtcacagcggcatctaccactgctcaggcacgggaagacaccgctacacatctgcaggagtgtccatcacggtgaaagagctgtttaccacgccagtgctgagagcatccgtgtcatctcccttcccggaggggagtctggtcaccctgaactgtgagacgaatttgctcctgcagagacccggcttacagcttcacttctccttctacgtgggcagcaagatcctggagtacaggaacacatcctcagagtaccatatagcaagggcggaaagagaagatgctggattctactggtgtgaggtagccacggaggacagcagtgtccttaagcgcagccctgagttggagctccaagtgcttggtccccagtcatcagctcctggttctgcttctggttctggtgttcgaccagttaacatcaccgagcccacactggaactgctgcacagcagctgcgaccccaacgccttccacagcaccatccagctgtattgcttcatctacggccacatcctgaacgacgtgtccgtgtcctggctgatggacgacagagagatcaccgacaccctggcccagaccgtgctgatcaaagaggaaggcaagctggcctctacctgcagcaagctgaatatcacagagcagcagtggatgagcgagagcaccttcacctgtaaagtgacctcccagggcgtggactacctggcccacaccagaagatgccccgaccacgaacccagaggcgtgatcacctacctgatcccccctagccccctggacctgtaccagaacggcgctcctaagctgacctgcctggtggtggacctggaaagcgagaagaacgtgaacgtgacatggaaccaggaaaagaaaaccagcgtgtccgccagccagtggtacaccaagcaccacaacaacgccaccacctccatcaccagcatcctgcccgtggtggccaaggactggatcgagggctacggctaccagtgcatcgtggaccaccccgacttccctaagcccatcgtgcggagcatcaccaagacccctggccagagatctgcccccgaggtgtacgtgttccccccacctgaggaagagtccgaggacaagagaaccctgacctgtctgatccagaacttcttcccagaggacatcagcgtgcagtggctgggcgacggcaagctgatctccaacagccagcacagcacaaccacccctctgaagtccaacggcagcaaccagggcttcttcatcttcagcagactggaagtggccaagaccctgtggacccagagaaagcagtttacatgccaagtgatccatgaggccctgcagaagcccagaaagctggaaaagaccatcagcaccagcctgggcaacacctccctgcgccctagttagctcgag

SEQ ID NO: 14 - protein, 613 aa, Artificial Sequence
  Synthetic Construct
HMEVVNATKAVITLQPPWVSIFQKENVTLWCEGPHLPGDSSTQWFINGTAVQISTPSYSIPEASFQDSGEYRCQIGSSMPSDPVQLQIHNDWLLLQASRRVLTEGEPLALRCHGWKNKLVYNVVFYRNGKSFQFSSDSEVAILKTNLSHSGIYHCSGTGRHRYTSAGVSITVKELFTTPVLRASVSSPFPEGSLVTLNCETNLLLQRPGLQLHFSFYVGSKILEYRNTSSEYHIARAEREDAGFYWCEVATEDSSVLKRSPELELQVLGPQSSAPGSASGSGVRPVNITEPTLELLHSSCDPNAFHSTIQLYCFIYGHILNDVSVSWLMDDREITDTLAQTVLIKEEGKLASTCSKLNITEQQWMSESTFTCKVTSQGVDYLAHTRRCPDHEPRGVITYLIPPSPLDLYQNGAPKLTCLVVDLESEKNVNVTWNQEKKTSVSASQWYTKHHNNATTSITSILPVVAKDWIEGYGYQCIVDHPDFPKPIVRSITKTPGQRSAPEVYVFPPPEEESEDKRTLTCLIQNFFPEDISVQWLGDGKLISNSQHSTTTPLKSNGSNQGFFIFSRLEVAKTLWTQRKQFTCQVIHEALQKPRKLEKTISTSLGNTSLRPS

SEQ ID NO: 15 - DNA, 1449 bp, Artificial Sequence
  Chimeric Protein: BBP-IgE
  CDS (1)..(1449)
catatgacttacaagctggtgatcaacggtaaaaccttgaagggtgagaccaccactgaggcagtcgacgccgccactgccgagaaggtctttaaacagtatgccaatgataacggcgtggacggcgagtggacctacgatgacgccactaagacattcactgtgactgaaaagcccgaggtgattgacgcgtccgaattgacacctgcggtgaccacctacaaactggttatcaacggcaagactctgaagggcgagaccaccacagaggcagtcgatgccgccaccgccgagaaggtcttcaagcaatatgccaacgacaacggggtggacggggagtggacctacgatgatgccaccaagaccttcaccgtgaccgagaagcccgaagtgatcgatgcgagtgaactgactcccgccgtgacaggttctgcttctggttctggtgttcgaccagttaacatcaccgagcccacactggaactgctgcacagcagctgcgaccccaacgccttccacagcaccatccagctgtattgcttcatctacggccacatcctgaacgacgtgtccgtgtcctggctgatggacgacagagagatcaccgacaccctggcccagaccgtgctgatcaaagaggaaggcaagctggcctctacctgcagcaagctgaatatcacagagcagcagtggatgagcgagagcaccttcacctgtaaagtgacctcccagggcgtggactacctggcccacaccagaagatgccccgaccacgaacccagaggcgtgatcacctacctgatcccccctagccccctggacctgtaccagaacggcgctcctaagctgacctgcctggtggtggacctggaaagcgagaagaacgtgaacgtgacatggaaccaggaaaagaaaaccagcgtgtccgccagccagtggtacaccaagcaccacaacaacgccaccacctccatcaccagcatcctgcccgtggtggccaaggactggatcgagggctacggctaccagtgcatcgtggaccaccccgacttccctaagcccatcgtgcggagcatcaccaagacccctggccagagatctgcccccgaggtgtacgtgttccccccacctgaggaagagtccgaggacaagagaaccctgacctgtctgatccagaacttcttcccagaggacatcagcgtgcagtggctgggcgacggcaagctgatctccaacagccagcacagcacaaccacccctctgaagtccaacggcagcaaccagggcttcttcatcttcagcagactggaagtggccaagaccctgtggacccagagaaagcagtttacatgccaagtgatccatgaggccctgcagaagcccagaaagctggaaaagaccatcagcaccagcctgggcaacacctccctgcgccctagttagctcgag

SEQ ID NO: 16 - protein, 480 aa, Artificial Sequence
  Synthetic Construct
HMTYKLVINGKTLKGETTTEAVDAATAEKVFKQYANDNGVDGEWTYDDATKTFTVTEKPEVIDASELTPAVTTYKLVINGKTLKGETTTEAVDAATAEKVFKQYANDNGVDGEWTYDDATKTFTVTEKPEVIDASELTPAVTGSASGSGVRPVNITEPTLELLHSSCDPNAFHSTIQLYCFIYGHILNDVSVSWLMDDREITDTLAQTVLIKEEGKLASTCSKLNITEQQWMSESTFTCKVTSQGVDYLAHTRRCPDHEPRGVITYLIPPSPLDLYQNGAPKLTCLVVDLESEKNVNVTWNQEKKTSVSASQWYTKHHNNATTSITSILPVVAKDWIEGYGYQCIVDHPDFPKPIVRSITKTPGQRSAPEVYVFPPPEEESEDKRTLTCLIQNFFPEDISVQWLGDGKLISNSQHSTTTPLKSNGSNQGFFIFSRLEVAKTLWTQRKQFTCQVIHEALQKPRKLEKTISTSLGNTSLRPS

SEQ ID NO: 17 - DNA, 864 bp, Artificial Sequence
  Chimeric Protein:  mSa-CD3Z
  CDS (1)..(864)
atgaagtggaaagccctttttaccgccgccattctgcaagcgcaattgccgatcactgaagccgcatcggccgaggccggtatcactggaacctggtacaaccagcacggatccacattcaccgtgaccgccggtgctgacggaaatctgaccggacagtacgagaatcgggctcagggcaccggttgtcagaactccccttacaccctcactgggagatacaacggcaccaagctggaatggagggtggaatggaacaactccaccgaaaactgccattcccgcactgagtggcgcggacagtatcaggggggagccgaagcgcggatcaacacccaatggaacctgacctacgagggcgggagcggacccgcgactgagcagggccaggatacgttcactaaggtcaagggcagcgcatcaggctcgggacagagctttggcctgctggatcccaaactctgctacctgctggatggaatcctcttcatctatggtgtcattctcactgccttgttcctgagagtgaagttcagcaggagcgcagacgcccccgcgtaccagcagggccagaaccagctctataacgagctcaatctaggacgaagagaggagtacgatgttttggacaagagacgtggccgggaccctgagatggggggaaagccgcagagaaggaagaaccctcaggaaggcctgtacaatgaactgcagaaagataagatggcggaggcctacagtgagattgggatgaaaggcgagcgccggaggggcaaggggcacgatggcctttaccagggtctcagtacagccaccaaggacacctacgacgcccttcacatgcaggccctgccccctcgctaa

SEQ ID NO: 18 - protein, 287 aa, Artificial Sequence
  Synthetic Construct
MKWKALFTAAILQAQLPITEAASAEAGITGTWYNQHGSTFTVTAGADGNLTGQYENRAQGTGCQNSPYTLTGRYNGTKLEWRVEWNNSTENCHSRTEWRGQYQGGAEARINTQWNLTYEGGSGPATEQGQDTFTKVKGSASGSGQSFGLLDPKLCYLLDGILFIYGVILTALFLRVKFSRSADAPAYQQGQNQLYNELNLGRREEYDVLDKRRGRDPEMGGKPQRRKNPQEGLYNELQKDKMAEAYSEIGMKGERRRGKGHDGLYQGLSTATKDTYDALHMQALPPR

SEQ ID NO: 19 - protein, 7 aa, Artificial Sequence
  Linker
GSASGSG